European Patent Specification EP 3 082 423 B1, published December 11, 2024. Title: CANCER TREATMENTS USING COMBINATIONS OF CDK AND ERK INHIBITORS. Applicant: SAHA, Saurabh. Application US 61/919,597. The sequence listing filed with the application follows.

SEQUENCE LISTING (18 sequences)

SEQ ID NO: 1 - DNA, 4454 bp, Homo sapiens
gaaacgtcccgtgtgggaggggcgggtctgggtgcggcctgccgcatgactcgtggttcggaggcccacgtggccggggcggggactcaggcgcctggggcgccgactgattacgtagcgggcggggccggaagtgccgctccttggtgggggctgttcatggcggttccggggtctccaacatttttcccggctgtggtcctaaatctgtccaaagcagaggcagtggagcttgaggttcttgctggtgtgaaatgactgagtacaaactggtggtggttggagcaggtggtgttgggaaaagcgcactgacaatccagctaatccagaaccactttgtagatgaatatgatcccaccatagaggattcttacagaaaacaagtggttatagatggtgaaacctgtttgttggacatactggatacagctggacaagaagagtacagtgccatgagagaccaatacatgaggacaggcgaaggcttcctctgtgtatttgccatcaataatagcaagtcatttgcggatattaacctctacagggagcagattaagcgagtaaaagactcggatgatgtacctatggtgctagtgggaaacaagtgtgatttgccaacaaggacagttgatacaaaacaagcccacgaactggccaagagttacgggattccattcattgaaacctcagccaagaccagacagggtgttgaagatgctttttacacactggtaagagaaatacgccagtaccgaatgaaaaaactcaacagcagtgatgatgggactcagggttgtatgggattgccatgtgtggtgatgtaacaagatacttttaaagttttgtcagaaaagagccactttcaagctgcactgacaccctggtcctgacttccctggaggagaagtattcctgttgctgtcttcagtctcacagagaagctcctgctacttccccagctctcagtagtttagtacaataatctctatttgagaagttctcagaataactacctcctcacttggctgtctgaccagagaatgcacctcttgttactccctgttatttttctgccctgggttcttccacagcacaaacacacctctgccaccccaggtttttcatctgaaaagcagttcatgtctgaaacagagaaccaaaccgcaaacgtgaaattctattgaaaacagtgtcttgagctctaaagtagcaactgctggtgattttttttttctttttactgttgaacttagaactatgctaatttttggagaaatgtcataaattactgttttgccaagaatatagttattattgctgtttggtttgtttataatgttatcggctctattctctaaactggcatctgctctagattcataaatacaaaaatgaatactgaattttgagtctatcctagtcttcacaactttgacgtaattaaatccaactttcacagtgaagtgcctttttcctagaagtggtttgtagacttcctttataatatttcagtggaatagatgtctcaaaaatccttatgcatgaaatgaatgtctgagatacgtctgtgacttatctaccattgaaggaaagctatatctatttgagagcagatgccattttgtacatgtatgaaattggttttccagaggcctgttttggggctttcccaggagaaagatgaaactgaaagcacatgaataatttcacttaataatttttacctaatctccacttttttcataggttactacctatacaatgtatgtaatttgtttcccctagcttactgataaacctaatattcaatgaacttccatttgtattcaaatttgtgtcataccagaaagctctacatttgcagatgttcaaatattgtaaaactttggtgcattgttatttaatagctgtgatcagtgattttcaaacctcaaatatagtatattaacaaattacattttcactgtatatcatggtatcttaatgatgtatataattgccttcaatccccttctcaccccaccctctacagcttcccccacagcaataggggcttgattatttcagttgagtaaagcatggtgctaatggaccagggtcacagtttcaaaacttgaacaatccagttagcatcacagagaaagaaattcttctgcatttgctcattgcaccagtaactccagctagtaattttgctaggtagctgcagttagccctgcaaggaaagaagaggtcagttagcacaaaccctttaccatgactggaaaactcagtatcacgtatttaaacatttttttttcttttagccatgtagaaactctaaattaagccaatattctcatttgagaatgaggatgtctcagctgagaaacgttttaaattctctttattcataatgttctttgaagggtttaaaacaagatgttgataaatctaagctgatgagtttgctcaaaacaggaagttgaaattgttgagacaggaatggaaaatataattaattgatacctatgaggatttggaggcttggcattttaatttgcagataataccctggtaattctcatgaaaaatagacttggataacttttgataaaagactaattccaaaatggccactttgttcctgtctttaatatctaaatacttactgaggtcctccatcttctatattatgaattttcatttattaagcaaatgtcatattaccttgaaattcagaagagaagaaacatatactgtgtccagagtataatgaacctgcagagttgtgcttcttactgctaattctgggagctttcacagtactgtcatcatttgtaaatggaaattctgcttttctgtttctgctccttctggagcagtgctactctgtaattttcctgaggcttatcacctcagtcatttcttttttaaatgtctgtgactggcagtgattctttttcttaaaaatctattaaatttgatgtcaaattagggagaaagatagttactcatcttgggctcttgtgccaatagcccttgtatgtatgtacttagagttttccaagtatgttctaagcacagaagtttctaaatggggccaaaattcagacttgagtatgttctttgaataccttaagaagttacaattagccgggcatggtggcccgtgcctgtagtcccagctacttgagaggctgaggcaggagaatcacttcaacccaggaggtggaggttacagtgagcagagatcgtgccactgcactccagcctgggtgacaagagagacttgtctccaaaaaaaaagttacacctaggtgtgaattttggcacaaaggagtgacaaacttatagttaaaagctgaataacttcagtgtggtataaaacgtggtttttaggctatgtttgtgattgctgaaaagaattctagtttacctcaaaatccttctctttccccaaattaagtgcctggccagctgtcataaattacatattccttttggtttttttaaaggttacatgttcaagagtgaaaataagatgttctgtctgaaggctaccatgccggatctgtaaatgaacctgttaaatgctgtatttgctccaacggcttactatagaatgttacttaatacaatatcatacttattacaatttttactataggagtgtaataggtaaaattaatctctattttagtgggcccatgtttagtctttcaccatcctttaaactgctgtgaatttttttgtcatgacttgaaagcaaggatagagaaacactttagagatatgtggggtttttttaccattccagagcttgtgagcataatcatatttgctttatatttatagtcatgaactcctaagttggcagctacaaccaagaaccaaaaaatggtgcgttctgcttcttgtaattcatctctgctaataaattataagaagcaaggaaaattagggaaaatattttatttggatggtttctataaacaagggactataattcttgtacattatttttcatctttgctgtttctttgagcagtctaatgtgccacacaattatctaaggtatttgttttctataagaattgttttaaaagtattcttgttaccagagtagttgtattatatttcaaaacgtaagatgatttttaaaagcctgagtactgacctaagatggaattgtatgaactctgctctggagggaggggaggatgtccgtggaagttgtaagacttttatttttttgtgccatcaaatataggtaaaaataattgtgcaattctgctgtttaaacaggaactattggcctccttggccctaaatggaagggccgatattttaagttgattattttattgtaaattaatccaacctagttctttttaatttggttgaatgttttttcttgttaaatgatgtttaaaaaataaaaactggaagttcttggcttagtcataattctt

SEQ ID NO: 2 - protein, 189 aa, Homo sapiens
MTEYKLVVVGAGGVGKSALTIQLIQNHFVDEYDPTIEDSYRKQVVIDGETCLLDILDTAGQEEYSAMRDQYMRTGEGFLCVFAINNSKSFADINLYREQIKRVKDSDDVPMVLVGNKCDLPTRTVDTKQAHELAKSYGIPFIETSAKTRQGVEDAFYTLVREIRQYRMKKLNSSDDGTQGCMGLPCVVM

SEQ ID NO: 3 - DNA, 1326 bp, Rattus norvegicus
gccgttcatggcggtttcggggtctccaacagcttctcaggttgaaatccaaaagcctcccgaggcggggtctgcggagtttgagatttttgcaggtgtgaaatgactgagtacaaactggtggtggttggagcaggtggcgttgggaaaagtgctttgacaatccagctaatccagaaccactttgtggatgaatatgatcccaccatagaggattcttaccgaaaacaagtggtgattgacggtgagacctgtctactggacatactggacacagctggacaagaggagtacagtgccatgagagaccaatacatgaggacaggcgaagggttcctctgtgtgtttgccatcaataatagcaaatcctttgcagatattaacctctacagggagcaaattaagcgcgtgaaagactctgatgatgtacccatggtgctggtagggaacaagtgtgacttgccaacaaggacagttgacacaaagcaagcccacgagctggccaagagttatggaattccattcattgaaacctcagccaagacccgacagggtgtggaggatgccttttacacgcttgtaagggagatacgccagtaccggatgaagaagctcaacagcagtgaggatggcactcaaggctgtatggggctgccctgtgtggtgatgtagtaagaccctttaaaagttctgtcatcagaaacgagccactttcaagcctcactgatgccctggttctgacatccctggaggagacgtgtttctgctgctctctgcatctcagagaagctcctgcttcctgcttccccaacttagttactgagcacagccatctaacctgagacctcttcagaataactacctcctcactcggctgtccgaccagagaaatgaacctgtttctccccagtagttctctgccctgggtttcccctagaaacaaacacacctgccagctggctttgtcctccgaaaagcagtttacattgatgcagagaaccaaactatagacaagcaattctgttgtcaacagtttcttaagctctaaggtaacaattgctggtgatttccccctttgcccccaactgttgaacttggccttgttagttttgggggaaatgtcaaaaattaatctcttcccgagaatagaattagtgttgctgattgcctgatttgcaatgtgatcagctatattctataagctggcgtctgctctgtattcataaatgcaaacatgagtactgacgtaagtgcatccctagtcttctcagctgcatgcaattaaatccaacgttcacaacaaaaaaaaaaaaaaaaaaaaaaaaa

SEQ ID NO: 4 - protein, 189 aa, Rattus norvegicus
MTEYKLVVVGAGGVGKSALTIQLIQNHFVDEYDPTIEDSYRKQVVIDGETCLLDILDTAGQEEYSAMRDQYMRTGEGFLCVFAINNSKSFADINLYREQIKRVKDSDDVPMVLVGNKCDLPTRTVDTKQAHELAKSYGIPFIETSAKTRQGVEDAFYTLVREIRQYRMKKLNSSEDGTQGCMGLPCVVM

SEQ ID NO: 5 - DNA, 4470 bp, Mus musculus
gggactggggcgccttgggcgcctagtgattacgtagcgggtggggccggaagtgccgctccctggcgggggctgttcatggcggtttcggggtctccaacagcttctcaggttgaagtccaaaagcctcccgaggcggggtctgcggagtttgaggtttttgctggtgtgaaatgactgagtacaaactggtggtggttggagcaggtggtgttgggaaaagcgccttgacgatccagctaatccagaaccactttgtggatgaatatgatcccaccatagaggattcttaccgaaagcaagtggtgattgatggtgagacctgcctgctggacatactggacacagctggacaagaggagtacagtgccatgagagaccagtacatgaggacaggcgaagggttcctctgtgtatttgccatcaataatagcaaatcatttgcagatattaacctctacagggagcaaattaagcgtgtgaaagattctgatgatgtccccatggtgctggtaggcaacaagtgtgacttgccaacaaggacagttgacacaaagcaagcccacgaactggccaagagttacggaattccattcattgagacctcagccaagacccgacagggtgtggaggatgccttttacacactggtaagggagatacgccagtaccgaatgaaaaagctcaacagcagtgacgatggcactcaaggttgtatggggctgccctgtgtgctgatgtagtaagacactttgaaagttctgtcatcagaaaagagccactttgaagctgcactgatgccctggttctgacatccctggaggagacctgttcctgctgctctctgcatctcagagaagctcctgcttcctgcttccccgactcagttactgagcacagccatctaacctgagacctcttcagaataactacctcctcactcggctgtctgaccagagaaatagacctgtctctcccggtcgttctctgccctgggttcccctagaaacagacacagcctccagctggctttgtcctctgaaaagcagtttacattgatgcagagaaccaaactagacatgccattctgttgacaacagtttcttatactctaaggtaacaactgctggtgattttcccctgcccccaactgttgaacttggccttgttggtttggggggaaaatgtcataaattactttcttcccaaaatataattagtgttgctgattgatttgtaatgtgatcagctatattccataaactggcatctgctctgtattcataaatgcaaacacgaatactctcaactgcatgcaattaaatccaacattcacaacaaagtgcctttttcctaaaagtgctctgtaggctccattacagtttgtaattggaatagatgtgtcaagaaccattgtataggaaagtgactctgagccatctacctttgagggaaaggtgtatgtacctgatggcagatgctttgtgtatgcacatgaagatagtttccctgtctgggattctcccaggagaaagatggaactgaaacaattacaagtaatttcatttaattctagctaatcttttttttttttttttttttttttggtagactatcacctataaatatttggaatatcttctagcttactgataatctaataattaatgagcttccattataatgaattggttcataccaggaagccctccatttatagtatagatactgtaaaaattggcatgttgttactttatagctgtgattaatgattcctcagaccttgctgagatatagttattagcagacaggttatatctttgctgcatagtttcttcatggaatatatatctatctgtatgtggagagaacgtggccctcagttcccttctcagcatccctcatctctcagcctagagaagttcgagcatcctagaggggcttgaacagttatctcggttaaaccatggtgctaatggaccgggtcatggtttcaaaacttgaacaagccagttagcatcacagagaaacagtccatccatatttgctccctgcctattattcctgcttacagacttttgcctgatgcctgctgttagtgctacaaggataaagcttgtgtggttctcaccaggactggaagtacctggtgagctctggggtaagcctagatatctttacattttcagacccttattcttagccacgtggaaactgaagccagagtccatacctccatctccttccccccccaaaaaaattagattaatgttctttatatagcttttttaaagtatttaaaacatgtctataagttaggctgccaactaacaaaagctgatgtgtttgttcaaataaagaggtatccttcgctactcgagagaagaatgtaaaatgccattgattgttgtcacttggaggcttgatgtttgccctgataattcattagtgggttttgtttgtcacatgatacctaagatgtaactcagctcagtaattctaatgaaaacataaattggataccttaattgaaaaaagcaaacctaattccaaaatggccattttctcttctgatcttgtaatacctaaaattctgaggtccttgggattcttttgtttataacaggatcttgctgtgtagtcctagctggcctcaaactcacaatactcttcctggatcaatctcccaagtgctgggattacaggcacattccaccacacacacctgactgagctcgttcctaatgagttttcattaagcaaattccccatcaccttgaaactaatcagaagggggaagaaacatttgctatgctcctgagtgctaacactgggatcattcacatggggtttgcattcctaggcaaactaaactgctgccttttacaacaaggctcagtcatcttcctgaagctgctgagaccagcacttggtcttgttttgttttaatatgtctatatgactggtggtggatccctaaatagtttattaattaaactccagttaaggagaaagttactcaccttgacccgtttgaccatatcccgtgtgtgtgtgtgtgtgtgtgtgtgtgtgtgtgtgtgtgtgtgtgtgcacgcgtatgtacgtacgtatgtatgtaggtatgtaggtggtttccagtataaacacagaaacaaatggagccaattcaggtttcagatgcccttactaacatatattcccacggggtgtgggttttggcacaacagtgacaaacttaaaagccaagtaagagccgggcgtggtggcgcacgcctttaatcccagcacttgggaggcagaggcaggcggatttctgagttctaggccatcctggtctacagtgagttccaggacagccagtgctacacagagaaaccctgtctcgaaaagccaaaaaaaaaaaaaaaaaaaaaaaaaaaaagccaagtaggtccagttggtatagtatcaaagtgtttttagagtaattagtgaaggtctgctttacctcaaagttgcagagcctctcttcctgagtttaagtgcctggccggcagtcacaaattaacatgttgctgtaaggcagttagttgaagctttgttcacacattggagagtatgaaaataaagtgttctaagagcgctgatactggatctgtgtaaacctggtaaatgccgtttgtccaggacttagcgtgtgtgagttggtagctcagtacgagtttactagttccgcagtgtgtacaatggaggcgggtttgttttagctggccacctgtagaatcagcctttaaactgctgtgaactttgtcatgacttgaatatgaagatagacaaaaactctgtaaagacaaatgtttgttttcccccttacagaacgtgtgagcttggttttatcttcctttgtatttagtcataacctctcaagctggcagctccgaccaaggatcagaagctgtgtgcgttccacctggtggaattagctcagctctatatgagaagtggagttaatggaaaacgtgttgactgggtggtttctatttaaaagagtgatgataattcttgaacagtagtttttattttgctatttctttaagctgactgatgtgccacaaaattattttaaggtatttgtgttttaagagtgttctcatgagattagttgtagatattttttaaaatacaactggtttttaaaatctgagtattgctctaagcaagtgtttagactcttacgggaaggtgggtggaagttgtttggcttccgtatttccatgcgtgccgtcagacataggtcagaacgccaactgtgcatcctgctgtttaaagacctcttggcctctgtgaccctcatgaaggggctgatattttaagttgactgtttgattgtaaattaatcctttctaatttttaaagacttgcttgactgttttccttgttaaataattttaaaaaaataaaaaactggaagttctttgcttaactgta

SEQ ID NO: 6 - protein, 189 aa, Mus musculus
MTEYKLVVVGAGGVGKSALTIQLIQNHFVDEYDPTIEDSYRKQVVIDGETCLLDILDTAGQEEYSAMRDQYMRTGEGFLCVFAINNSKSFADINLYREQIKRVKDSDDVPMVLVGNKCDLPTRTVDTKQAHELAKSYGIPFIETSAKTRQGVEDAFYTLVREIRQYRMKKLNSSDDGTQGCMGLPCVLM

SEQ ID NO: 7 - DNA, 570 bp, Cavia porcellus
atgactgagtataaactggtggtggttggagcaggtggtgtcgggaaaagtgcactgaccatccagctaattcagaaccactttgtcgatgaatatgatcccaccatagaggattcttaccgaaaacaggtggttatagatggtgaaacttgtctgttggatattctggatacagctggacaagaggagtacagtgccatgagagaccaatacatgaggacaggcgaaggcttcctctgtgtgtttgccatcaataatagcaaatcatttgcagatattaacctctacagggagcagattaaacgagtaaaagactcagatgatgtacctatggtgctggtagggaacaagtgtgatttgccaacaaggactgttgacacaaaacaagcccatgaactggccaagagttacgggattccattcattgaaacctcagccaagaccagacagggtgttgaagatgcattttacacactcgtaagagaaatacgccagtacagaatgaaaaaactcaacagcaatgatgatgggactcaaggttgtatggggttgccatgtgtggtgatgtaa

SEQ ID NO: 8 - protein, 189 aa, Cavia porcellus
MTEYKLVVVGAGGVGKSALTIQLIQNHFVDEYDPTIEDSYRKQVVIDGETCLLDILDTAGQEEYSAMRDQYMRTGEGFLCVFAINNSKSFADINLYREQIKRVKDSDDVPMVLVGNKCDLPTRTVDTKQAHELAKSYGIPFIETSAKTRQGVEDAFYTLVREIRQYRMKKLNSNDDGTQGCMGLPCVVM

SEQ ID NO: 9 - DNA, 1220 bp, Cavia porcellus
gttccggggtcctcaacgtttctcagggttgagattctatatccttttgaagctggggcggcagagcttgaggttcttgctggtgtgaaatgactgagtataaactggtggtggttggagcaggtggtgtcgggaaaagtgcactgaccatccagctaattcagaaccactttgtcgatgaatatgatcccaccatagaggattcttaccgaaaacaggtggttatagatggtgaaacttgtctgttggatattctggatacagctggacaagaggagtacagtgccatgagagaccaatacatgaggacaggcgaaggcttcctctgtgtgtttgccatcaataatagcaaatcatttgcagatattaacctctacagggagcagattaaacgagtaaaagactcagatgatgtacctatggtgctggtagggaacaagtgtgatttgccaacaaggactgttgacacaaaacaagcccatgaactggccaagagttacgggattccattcattgaaacctcagccaagaccagacagggtgttgaagatgcattttacacactcgtaagagaaatacgccagtacagaatgaaaaaactcaacagcaatgatgatgggactcaaggttgtatggggttgccatgtgtggtgatgtaacaagatatttaacaaagttctatcagaaaagagccactttcaagctgcactgataccctggtcctgacttccctggaggagaagtatccctgttgctctcttcatctcagagaagctcctgctgtttgtccacctctcagtgtatgagcacagtctctgcttgagaacttctcagaataactacctcctcacttggttgtctgaccagagaaatgcacctcttgttaattccccaataattttctgccctgggctctccccaacaaaaaacaaacacttctgccatccaaaaagcaacttggtctgaaacagaaccaaactgtagattgaaattctcttaaaaagtcttgagctctaaagttagcaaccgctggtgatttttattttcctttttatttttgaacttggaactgacctatgttagattttggagaaatgtcataaagtactgttgtgccaagaagataattatgttgctgaatggttgatttatagtgttatcagctatattttacaaactggcatctgctctgtattcataaatacaaaaatgaagccagg

SEQ ID NO: 10 - protein, 189 aa, Cavia porcellus; identical to SEQ ID NO: 8

SEQ ID NO: 11 - DNA, 1307 bp, Canis lupus
tgattacgtagcgggcggggccggaagtgccgctccctagtgggggctgttcatggcggttccggggtctccaacctttctcctagttgtggtcctaaatacgtcggaagcggaggcggcgaagcttgaggttcttgctggtgtgaaatgactgagtacaaactggtggtggttggagcaggtggtgttgggaaaagcgcactgacaatccagctaatccagaaccactttgtagatgaatatgatcccaccatagaggattcttaccgaaaacaggtggttatagacggtgaaacctgtctgttggatatactggatacagctggtcaagaagagtacagtgccatgagagaccaatacatgaggacaggcgaaggcttcctctgtgtatttgccatcaataatagcaaatcatttgcagacattaacctctacagggaacagattaagcgagtaaaagattcagatgatgtacctatggtgctagtaggaaacaagtgtgatttgccaacaaggacagttgacacaaaacaagcccatgaactggccaagagttatgggattccattcattgaaacctcagccaagaccagacagggtgtcgaggatgccttttacacactggtaagagaaatacgtcagtaccgaatgaagaaactcaacagcagtgatgatgggactcaaggttgtatggggttaccatgtgtggtgatgtaacaagacacttttaaagttctagcatcagaaaagagccactgtcaagctgcactgacaccctggtcctgacttccctggaggagaagtattcctgttgctatcttcagtctcacaaagaagctcctgctacttccccaactctcagtagatcagtacaatgttctctatttgagaagttctccgaacaactacctcctcacttggttgtctgaccagagaaatgaacctcttgttccttcccgctgtttttccaccctgaattctcccccaacacacataaacaaacctctgccatcccaggtttttcatctgaaaaataattcatgctctgaaacagagaacaaaactgtagacatgaaattctgtaggaaacaaggtcttgagctcaaaagtagcaactgctggtgacctttttttcccccctttttactgttgaacttggaactatgttggtttttggagaaatgtcataagttactgttttgctgagaatatagttaagttgacatttggtttgtttgtaatatcattagctattttctataaattggcatctgctctgcattcataaatacacgagtgaattctga

SEQ ID NO: 12 - protein, 189 aa, Canis lupus; identical to SEQ ID NO: 2

SEQ ID NO: 13 - DNA, 3104 bp, Felis catus
aaaaaataaataaatttaagaaaccattttaaaattatgcacagttgcagcctggaaaacttaaggtggcgccttatagtatcaatcttaggagctttatttggtgcatttaacgcaactggtaattgcaaaatccacttcgcctgtgtaagtgaaaaatatagactgttatcttgttggccctatgaaattctgcacttggtatttagcatatactctaccttcattactatctggcaagatgttctgccttagcactcagttgcattcttttccttttctttcctgttcattatgctttaattctgaggaccatatgagggtagaatatattaaaaattacaaaaattataaaaatttgtataggcaaaccatttccttaagttgatggccaaatgttaaaatgttatttttcatatcatttataatcttgtcacagtccacttaacgaagtttggttagatttcagtgaaaattatcttccagagtagtttttttttttttttcctgggattagggaggggggtaactttactgcaattagtatgtatggtgcagaatttcatgcaaatgaggtgtgccagcagtgtggtaatttaatcgtatttaaacaaaaacaaacaaaaaaaaaacgaatgcacaaacttgctgctgcttagatcactgcagcttctaggacccagtttcttttactgatttcaaaacaaaacaaaacaaaaaaataaaaaaagttgtgcctgaaatgaatcttgttttttttataagtagccgcctggttcctgtgtcctgtgaaatacaggcacttgacccttggtgtagcttctgttcgactttatatcacgggaatggattggtctgatttcttggccctcatcttgaattggccacatccagggtccctggccagtggactgaaggctttgtctaagaggacaagggcagctcaggggatgtgggggagggcgcttttatcttccccgttgtcgtttgaggttttgatcttctctgggtaaagaggccgtttatctttgtaaacacaaaacatttttgctttctccagttttctgttaatggcgaaagaatggaagcgaataaagttttactgatttttgagactctagcacctagcgctttcatttttgaaacgtcctgtgtgggaggggcgggtctgggtgcggcccgccgcgtgactcctgagtcgggggcccacgtggctggggcggggactcggacgccccgggcgccgactgattacgtagcgggcggggccggaagtgccgctccctagtgggggctgttcatggcggttccggggtctccatcctttttcccagttgttctaaatcagtcggaagcggaggcagcgaagtttgaggttctcgctggtgtgaaatgactgagtacaaactggtggtggttggagcaggtggtgttgggaaaagcgcactgacaatccagctaatccagaaccactttgtagatgaatatgatcccaccatagaggattcttaccgaaaacaggtggttatagacggtgaaacctgtctgttggacatactggatacagctggtcaagaagagtacagtgccatgagagaccaatacatgaggacaggcgaaggcttcctctgtgtatttgccatcaacaatagcaaatcatttgcagatattaacctttacagggaacagattaagcgagtaaaagactccgatgatgtacctatggtgctagtaggaaacaagtgtgatttgccaacaaggaccgtcgacacaaaacaagcccacgaactggccaagagttatgggattccattcattgaaacctcagccaagaccagacagggtgttgaagatgccttttacacactggtaagagaaatacgtcagtaccgaatgaagaaactcaacagcagtgatgacgggactcaaggttgtatggggttaccgtgtgtggtgatgtaacaagatacttttaaagttctagcatcagaaaagagccactgtcaagctgcactgacaccctggtcctgacttccctggaggagaagcgttcctgttgctattttcagtttcacaaagaagctcctgctatttccccaactctccgtagatcagtacattattctctgtttgagaagttctccgaataactacctcctcacttggttgtctgaccagagaaatgaacctcttgttactccccactgtttttccaccctggttctcccccagcacatataaacaaacctcccaggtttttcatctgaaaagtaattcatgctctgaaacagagaaccaaactgtagacatgaaattctgtaggaaacaatgtcttgagctctaaagtagcaactgctggtgactttttttttttttttttcctttttactgttgaacttggaactatgttggtttttggagaaatgtcgtaagttactgttttgctgagtatatagttaagtttaccattcggtttgtttgtaatgtcattggctatactctgtacctggcatctgctctgcattcataaatacaaaagtgaattctgacttttgagtctatcctagtgttctcaacttccacataattaaatctaacttttgcagcaaagtgcctttttcctagaagtggtttgtagatttgctttataatactttggtggaatagatgtctcaaaaaccattatacatgaaaatgaatgtctgagatacgtctatgatctgtctacctttgagggaaaaatataccgacataatagcagatgccatgtcttacgtgtatgaagttggatttccagagacctgatttgggtctcttccaagagaaagatgaaactggaaacaattatgaataacttcacttaatttttacctaatctctacttcggggtgggagggcagggagtaggttaccacttacaaaatatatgcaatttgtttcttctagcttactgataatgaacttccattcttatttaaatttaggtcatatcctaaagctttacatttgcaggtgttcgaaattgtaagtttaatgcagttttatttaatagctatgatcaatgattttcaagcctcagatgtattaacggacacattttcact

SEQ ID NO: 14 - protein, 189 aa, Felis catus; identical to SEQ ID NO: 2

SEQ ID NO: 15 - DNA, 4283 bp, Bos taurus
ggccgctccctagtgggggctgttcatggcggttccggggtctcccaacaattttcccggttgtggtcgtaatctatccgaagtggaggcagtggagctagaggttcttgctggtgtgaaatgactgagtacaaactggtggtggttggagcaggtggtgttgggaaaagtgcactgacaatccagctaatccagaaccactttgtagatgaatatgatcccaccatagaggattcctaccgaaaacaggtggttatagatggtgaaacctgtctgttggacatactggatacagctggacaagaggagtacagtgccatgagagaccaatacatgaggacaggcgaaggcttcctttgtgtgtttgccatcaataatagcaaatcatttgcagatattaacctctacagggaacagataaagcgtgtaaaggactcggatgatgtacctatggtgctagtaggaaacaagtgtgatttgccaacaaggacagttgacacaaaacaagcccatgaactggccaaaagttatgggattccattcattgaaacctcagccaagaccagacagggtgttgaagatgccttttacacactggtaagagaaatacgtcagtaccgaatgaaaaagctcaacagcagtgatgatggcactcaaggctgtatggggttgccgtgtgtggtgatgtaacaagatacttttaaagttctcacatcagaaaagagccactgtcaagctgcactgacaccctggtcctgacttccctggaggagaagtattcctgttgctatcttcagtttcaaaaagaagctcctgctatttccccaactctcagtagatcaatataatattctctatttgagaagttctcaagaataactacctcctcacttggttgtctgaccagagaattgaacctcttgttactcccagtatttttccaccctgggttctcccccagcacacacaaacgcacctctgccacccaggtttttcatctgaaaagcaattaatactctgaaacagagaaccaaactgtagaaacatgaaattctgtagaaaacaatgtcttgagctctaaagtagcaactgctggtgattttttttttttttttttcctttttattgttgaacttggaactatgttggtttgtggagaaatgtcataaattactgttttgctgagaatatagttaatgttgctctctggtttgtttgtaatgttatcagctatattctataaactggcatctactctgtatttagaaatacaaaaatgaatactgaccttttgagtctaccctcatcttctcgactttcttgtaattaaatgtaactttcacgatgaagtgccttttgcctgggagtgactcgtagacttcctttaaaatacttcagtggaatagatgtctcagaaactgttatacataagaataaatgtctgagatatgtctatgacccatctagctttgagggaaagatataccaatatgatagcagatgccatttcttacatctataacgttgattttctggagacctattttggggctctccgagagaaagatgagactataaatgattaggaataatttcacttaatttttacataacctccactttttgttttgtagtttactacctgcaaaacatataatttgattccttttagcttacagataatctaatgttaaatgaacttccattcatattttaatttggatcatatcaggaagtctacatttgcaggtgttcaaaaattgtaaaagtgtgatgcagttttatttaatagctgtgatcaatgattttcaagcctcaaatatgttaatagacacattttcactgtatatcatggtattaataattattgatgtatataattgtccttggtccccttctctgttcatcacctcatggcaatggcttgattaattatttcagctgagtaaagcatggtgctaatagaccagggtcacagtgtcaaaacttcagtgagccagtaagcatcacagagaaagaaattctttcacatttgctcaccattaactccagctaatagttttgccagatgtgtgtggttagtcctgcaaggaaaggagaagtcagttaatacaaattcttaaccaggactggaaaaacttgttttcctgagaagggtcagcttagaagtctttatctggactctatttttagccacatggaaatcaaattaagctgatcttttttctcaagtttttgagagtgaggatgcctcagatcaacatttttaaaatattctttattcttacgttcttttaagggtttaaaacaacgttgagtaattagtctgggcataccaggtaacaagctgataagtttgtgctgaacaagaagtagcctttggattgaaattgctgttttgagaagggatagaaaatataattaataattatgagacttgacttttctatttgcagataatatcctgataattctgatgaaaatagacttggataatttttgataaaagaatcgttccaaaatggccacttgctgttcttgtcttctaatgtgtaaatacttactgaggtcctcttctaatatgagttgtcatttattaagcaaattccacattgccttgaaatgaattcggaagagaagaaaaagtcatagtatacccagagaatgaaaaatccagagaattgtgctccttagtgttaattctgaagccttcgtagtccacacccatagacagaaactctctgccactttgcttctgctcctcttggagcattgcgctgtcatttccttgaggatagattgaggcttgtcaactcagttgtattgtcttcctcctcttcctcttgtctgtgtgactgacagtgtgactcttactaatgtcagatgcggggatgcggggaggtgggggggagtagctcattttaggctcttgcaccctttaccgttgtatgtgtgtgtcttttagttttctcaagaatgttctaagcacagaagtatctaaatggggccaaaattcagacttgaaaatgttcttttaatagcttcttaaaaagttacactttggtgtgaattttggcaggatagagtgacaaactcttaaacgctgaataacttcagttagtgtgttatagtttttagaatatgtttgtgattgctgaaaacaattatagtttacctcaaaatctgaaagtctctttccccaagttaagtgcctggccagctgtcaaagattacatattactttatgtttgtttgttttttaaaggttgcacattcaagattgtgaaaataaggtgttctgtctgaaagctaccatgcctgtctgtaaatgaatccactgagtgctgtacttgttccaacagcttactacagaatgctacttggtaatatcatactcgttacagttttcacttcaggagtgtactaggtagaatgatcctgtgtgtattgtagtgggctccatgtttagtcttttcagcatcctttaaactgctgtgaatttttgtcttgacttgaaagcaaggatagagaaacactttaaagagatactttgggtttttttccattccagaattggtgagcatagttagattttgctttacatttacagtcatgaactcttaagctggcagctacaaccaagaaccaaaagagggtgcattctgcttcttgtaattcatctttgctaataaattatgagaagcaaagataattaattagagaaactattttatttgggtggtttctataaacaagggactataattcttaaacattatttttcatttttgctgtttctttaagaaacctaatgtgccacaacattattttaaggtgtttcttaaaagaattgtttttaaaagtgttctcattttcagagtaattgtagatatatttcaaaatataactgataatttttaaaggcctgagtactgacctaagaagcagttgtatgaattctctggggggaagggaggagctcagtgaaagttgtatgacttttatatttctgtgccatcaaataaaggtaaaaatgtcttttgtgcagttttgctgttcaaacagaaactattggcctccttggccctaaatgaaagggctggtattttaagttgactattttattgtaaattaatccatcttaatttttttaaatttggttgaatgttctcttgttaaatgtttaaaaaataaaaactggaagttctttgcttagtcataaaaaaaaaaaaaaaaaaaaaaaaaaaaaaaaaaaaaaaaaaaaaaataaaaaaaaaaaaaaa

SEQ ID NO: 16 - protein, 189 aa, Bos taurus; identical to SEQ ID NO: 2

SEQ ID NO: 17 - DNA, 4825 bp, Gallus gallus
gcgccgggaccggaagccggaagctttgcagaagggtgttccgcgttcgcggtgcgggagcggtcagccggggtggcggggctggggccggccggggcaggcggctccgcgctccgcactgggccgctgggagggcgatgactgaatacaagctggtggtggtgggagctggcggcgtcgggaagagcgcgttgaccatccagctcatccagaaccacttcgtggacgagtacgaccccaccatcgaggattcgtacagaaagcaggttgtcatcgatggagagacgtgcttgttggacattctggacactgcaggacaggaagaatacagtgctatgcgtgatcagtacatgagaactggggaaggattcctttgtgtgtttgccattaacaacagtaaatcattcgctgatattaacctttacagagagcaaatcaagagagtgaaagattcagacgatgtgccaatggtgctggtggggaataagtgcgatttgccaacaaggacagtagacaccaaacaggctcaagagttagcaaaaagctacggcattcccttcatagagacatcagccaaaacgagacagggtgtggaagatgcgttttacacactggtgagggagattcggcagtaccggatgaaaaagctcaacagcaacgaagatgggaatcagggctgtatggggttgtcctgcattgtgatgtgataagatgccaggttcagatgtagctgctggacaagtctcgatgctactgtattgtgtctcatgctgatgccctgcagtattttggtgccagcgaccagactcttggtaccagttaattagctcaggatcctttcctgtgctccatctgaagaaaacatctctggtatctacctccttgctcagctcacagagcagtcatatctcttggtgtactgggattcttttctagctgtgttgtctgggtttgttcaagaagaaaaccagtcacaagaaaagtgaattacagagactaaatgctgtgaaaaagatcacactttacctccagagtaaaagctagaagtggcgtttgacccctttgcattggattcagatttgcggtgttgtcagaggagtggcagaagtaattttgccattacaaaggtttctgtcaccagtcggattggtatctgctgtctgtgcacccacacagtgtatctgcaacatctgcattgtgccagaagtatcacttaactgatgaactgatcctttatttttctgtaataaaaaggagatatctttgctaacttaagtgcctgtttgctcagaaggttggaggttgtatgctgttcccttgggctgaggagaaccccaaggatgaatttcttgggtgctcattgtcttgagcaggcaagttttgtgtgggtgatctcttttcatggcaggatattaaaatgggaatttgtagtctggaagatggagcagctgtttgtgagactcttgagttagggagagaaatgtataccacgtctgttctcgatccatcagaatggatccatccacctctttgtgtgtggaactgtgtatagtctgtattggttttctacagcacttggatctctttggaccaaattagcgagctgttcattttaacataactgccagtatttatagacaatttcttacggacagataatgaatttagaaactggaggttactttgggcagctgttcctcagctctgtctgtaacttgcaaattattctgagttattttctgcagaacctccttccttatcacgggaggagcctgggagttgaggttgactgtaattgggtcaatggttgtcacagacttaaggtgtccaggctgattggaggaggcactgagccctaacagagcactgagctgacttctaattgcagcatccttgcaaaatgaggaagggagttcagtgatgtctgcactgaagatgtatgatacactgatagcagttctgggtatgttgtaacagcttcaaagtagaaccgcagtactgcgtgagctgtgtgacttcttcctagaacacagcactgtcaccccatatggttgggacgtgcaggtgagaccaacacctaccaggttccctggcgtaccgtggccttctcagttcttgtgccagtgatactgggttctgttctgtggtgtcagacagcgtcctgtagcaaagctgaattcccacttagtctggtgagagaataaagagccatcagccaacagagggagcgttcattctgctggagcagtgcgagctgtaagcattacgagaggcgtagtttcagtttgttgcagtcaggttcctatattttcaaagctgaaatcagaaataagtaaatacggagaaaataagctgttgcttttaatgctctttcctccactaattgtactcttaattttcttcttgggaggccgaggatccatctgcataactttagctgtgatgctccagataagtgtttagaattcattttatctttgactgatgggactgataagaagttaacgcacaatatttttacatacaacatcgttttccagtgacctcctgagcggtgggaagcattatgggatagcaccggctgtgactcgagttcatttgaaggcgatctcttgcctgcaggttaaatgggacggagtcagaatcactgtgagccgtctgtaatcagcaaacagtctgtgggcttttcttactgtgttctctctgtttgccttagtttggtgcaggaagagttccttgtgacagcgtcctttgaggtgtgttgcaggagctgaccatttgctccttgagctgtgtgatgaactgttgtccacttaatggagttacagaagcagcttctgggagtcgcatctggtcgcatacattcagtgttttgggaagctgtcagtgtggtgtttgcactgtgtttgaatggtgttcatggtgggtctgttatgctcctggatgatttggggagatgtggggctgcttccgtggcagacaggatcagctcagggcgctgctgcctatggctgtgggaaacctcacagttggtgtttgaatagtggccaagtatgtcaattaaaaatacattttgaagggaggtttgtcatagctctgtactttggcatgctctgcttactgaaaacatactagctgtagctcaaaaaaagttgtgaatcctcagaataatacaggagctggcaattgtggctgctttctctttgtgttccttttctcttgggttggatgaagctttaaaaaggaaggagccctggtgagggttggtcagtgtgcatttcattcttggaaccagagaggaagttgcatcaactttcaggacgctgcagagctcacttgcacaggtggtgctccagtctatgtgatttttggggtcaaatcttgagatgatcttacaaaatcagattttgtacccatcatgagcatgaggtgagtggttgtgctcggtttctagctgcatgtatgtatacagacacgtgtatgcagacatgtctatgtgtgagtagttcgagtcagtcaaggttactggcagcacctaaagcgtatgcaccacataatgcatgcaggcaaaagtcctatcttaggagccatctcttcatgggtttgggtttatataggcagtatttttaaacagaatatccgaagcactttctggagttctgtggtaatgcagtgacacctatttggatgaaggaagatgtgtctgaggagcacgtaagcagatttgctgccctaacagagaggttttggtaaccgtggaaaaggttttctcctggatctgtgtgtgctcttggtgagctgcaatccatgacagggcacaaccagatgagaaggaaacccggccatcccatgcttgagcacagctctgactcagtagttccaccagatgtgccctttcagtcaaagtgttctgatctcttagagctttctgtagttcaagttaccactcactctccagcttgctcggttaatgtctgttggcggcgttgagttggacttgggaaaggtgtgtgtggtaggaacaagcagagtgtgatgtgcttctgttatcaggacttaagctagagtggttggcagataggaaatgcagctattccttgaaagcaagcagatcatggatggtcagccaaactgccctggctttggtgggagctgcactgcagaaggaccaaaccccaacaagatttggcacatttgtttagaagataagcacagatggttttgcacaaggcagctcctcataatggtggctttgtagatttagtccaaatgttcttatttagatctagcagcacatcactgtgtccgtgcccatctaacctcgctatcctaagtagagcagaccccaaacaaccttgttcaaaaactaccagtgcaaataactgaactaaatatttgttactgctgactgagaacagctgttcgagtgtagcattgtggcttgttaatgtgagtgccccaactctatggtcttattaaagaaacccaaacattgctcagattttgttcttattgtcatcataagacttgaatagtgatggtaatgcttacgtagacgtgtcttgtgagtgcacttcagtgatttagaaagaactggatttcaagcaactttggacctgtggggggagggagattaatgaaggtttgaatcacattctaattctatgtacagtccttcattactccacaagcctaaatcctatacagcctccaggatagctggaaactgttgagatctggactttttttttttaatccaagggctaacttgttgtaacttggtataattatctgctttcggaaatgcatctctgttggtttgaaa

SEQ ID NO: 18 - protein, 189 aa, Gallus gallus
MTEYKLVVVGAGGVGKSALTIQLIQNHFVDEYDPTIEDSYRKQVVIDGETCLLDILDTAGQEEYSAMRDQYMRTGEGFLCVFAINNSKSFADINLYREQIKRVKDSDDVPMVLVGNKCDLPTRTVDTKQAQELAKSYGIPFIETSAKTRQGVEDAFYTLVREIRQYRMKKLNSNEDGNQGCMGLSCIVM